European Patent Application EP 4 591 941 A2, published July 30, 2025. Title: BISPECIFIC ANTIBODY AND USE THEREOF. Applicant: KEYMED BIOSCIENCES CO., LTD. Application EP. The sequence listing filed with the application follows.

SEQUENCE LISTING (95 sequences)

SEQ ID NO: 1 - protein, 306 aa, Homo sapiens
QSIKGNHLVKVYDYQEDGSVLLTCDAEAKNITWFKDGKMIGFLTEDKKKWNLGSNAKDPRGMYQCKGSQNKSKPLQVYYRMCQNCIELNAPEAAGGPSVFLFPPKPKDTLMISRTPEVTCVVVDVSHEDPEVKFNWYVDGVEVHNAKTKPREEQYNSTYRVVSVLTVLHQDWLNGKEYKCKVSNKALPASIEKTISKAKGQPREPQVCTLPPSRDELTKNQVSLSCAVKGFYPSDIAVEWESNGQPENNYKTTPPVLDSDGSFFLVSKLTVDKSRWQQGNVFSCSVMHEALHNHYTQKSLSLSPGK

SEQ ID NO: 2 - protein, 339 aa, Homo sapiens
QDGNEEMGGITQTPYKVSISGTTVILTCPQYPGSEILWQHNDKNIGGDEDDKNIGSDEDHLSLKEFSELEQSGYYVCYPRGSKPEDANFYLYLRARVCENCMEMDAPEAAGGPSVFLFPPKPKDTLMISRTPEVTCVVVDVSHEDPEVKFNWYVDGVEVHNAKTKPREEQYNSTYRVVSVLTVLHQDWLNGKEYKCKVSNKALPASIEKTISKAKGQPREPQVYTLPPCRDELTKNQVSLWCLVKGFYPSDIAVEWESNGQPENNYKTTPPVLDSDGSFFLYSKLTVDKSRWQQGNVFSCSVMHEALHNHYTQKSLSLSPGKGSGLNDIFEAQKIEWHE

SEQ ID NO: 3 - protein, 305 aa, Macaca fascicularis
QSFEENRKLNVYNQEDGSVLLTCHVKNTNITWFKEGKMIDILTAHKNKWNLGSNTKDPRGVYQCKGSKDKSKTLQVYYRMCQNCIELNAPEAAGGPSVFLFPPKPKDTLMISRTPEVTCVVVDVSHEDPEVKFNWYVDGVEVHNAKTKPREEQYNSTYRVVSVLTVLHQDWLNGKEYKCKVSNKALPASIEKTISKAKGQPREPQVCTLPPSRDELTKNQVSLSCAVKGFYPSDIAVEWESNGQPENNYKTTPPVLDSDGSFFLVSKLTVDKSRWQQGNVFSCSVMHEALHNHYTQKSLSLSPGK

SEQ ID NO: 4 - protein, 330 aa, Macaca fascicularis
QDGNEEMGSITQTPYQVSISGTTVILTCSQHLGSEAQWQHNGKNKEDSGDRLFLPEFSEMEQSGYYVCYPRGSNPEDASHHLYLKARVCENCMEMDAPEAAGGPSVFLFPPKPKDTLMISRTPEVTCVVVDVSHEDPEVKFNWYVDGVEVHNAKTKPREEQYNSTYRVVSVLTVLHQDWLNGKEYKCKVSNKALPASIEKTISKAKGQPREPQVYTLPPCRDELTKNQVSLWCLVKGFYPSDIAVEWESNGQPENNYKTTPPVLDSDGSFFLYSKLTVDKSRWQQGNVFSCSVMHEALHNHYTQKSLSLSPGKGSGLNDIFEAQKIEWHE

SEQ ID NO: 5 - protein, 109 aa, Homo sapiens
QAVVTQEPSLTVSPGGTVTLTCRSSTGAVTTSNYANWVQQKPGQAPRGLIGGTNKRAPWTPARFSGSLLGGKAALTLSGAQPEDEAEYYCALWYSNLWVFGGGTKLTVL

SEQ ID NO: 6 - DNA, 327 bp, Homo sapiens
  source 1..327: mol_type = other DNA
caggctgtggtcacacaagagcctagcctgacagtgtctcctggcggcacagtgaccctgacctgtagatcttctacaggcgccgtgaccaccagcaactacgctaattgggtgcagcagaagcccggccaggctcctagaggactgatcggcggaacaaacaagagagccccttggacacccgccagattctctggatctctgctcggcggaaaggccgctctgacactttctggtgctcagcctgaggacgaggccgagtactattgtgccctgtggtacagcaacctgtgggtgttcggcggaggcaccaaactgacagttctg

SEQ ID NO: 7 - protein, 14 aa, Homo sapiens
RSSTGAVTTSNYAN

SEQ ID NO: 8 - protein, 8 aa, Homo sapiens
GGTNKRAP

SEQ ID NO: 9 - protein, 9 aa, Homo sapiens
ALWYSNLWV

SEQ ID NO: 10 - protein, 109 aa, Homo sapiens
QAVVTQEPSLTVSPGGTVTLTCRSSTGAVTTSNYANWVQEKPGQAPRGLIGGTNKRAPWTPARFSGSLLGGKAALTLSGAQPEDEAEYYCALWYSNLWVFGGGTKLTVL

SEQ ID NO: 11 - DNA, 327 bp, Homo sapiens
  source 1..327: mol_type = other DNA
caggctgtggtcacacaagagcctagcctgacagtgtctcctggcggcacagtgaccctgacctgtagatcttctacaggcgccgtgaccaccagcaactacgctaattgggtgcaggagaagcccggccaggctcctagaggactgatcggcggaacaaacaagagagccccttggacacccgccagattctctggatctctgctcggcggaaaggccgctctgacactttctggtgctcagcctgaggacgaggccgagtactattgtgccctgtggtacagcaacctgtgggtgttcggcggaggcaccaaactgacagttctg

SEQ ID NO: 12 - protein, 109 aa, Homo sapiens
EAVVTQEPSLTVSPGGTVTLTCESSDGAVTTSNYANWVQEKPGQAPRGLIGGTNKEAPWTPARFSGSLLGGKAALTLSGAQPEDEAEYYCALWYSNLWVFGGGTKLTVL

SEQ ID NO: 13 - DNA, 327 bp, Homo sapiens
  source 1..327: mol_type = other DNA
gaggctgtggtcacacaagagcctagcctgacagtgtctcctggcggcacagtgaccctgacctgtgagtcttctgacggcgccgtgaccaccagcaactacgctaattgggtgcaggagaagcccggccaggctcctagaggactgatcggcggaacaaacaaggaggccccttggacacccgccagattctctggatctctgctcggcggaaaggccgctctgacactttctggtgctcagcctgaggacgaggccgagtactattgtgccctgtggtacagcaacctgtgggtgttcggcggaggcaccaaactgacagttctg

SEQ ID NO: 14 - protein, 14 aa, Homo sapiens
ESSDGAVTTSNYAN

SEQ ID NO: 15 - protein, 8 aa, Homo sapiens
GGTNKEAP

SEQ ID NO: 16 - protein, 109 aa, Homo sapiens
QAVVTQEPSLTVSPGGTVTLTCESSDGAVTTSNYANWVQEKPGQAPRGLIGGTNKEAPWTPARFSGSLLGGKAALTLSGAQPEDEAEYYCALWYSNLWVFGGGTKLTVL

SEQ ID NO: 17 - DNA, 327 bp, Homo sapiens
  source 1..327: mol_type = other DNA
caggctgtggtcacacaagagcctagcctgacagtgtctcctggcggcacagtgaccctgacctgtgagtcttctgacggcgccgtgaccaccagcaactacgctaattgggtgcaggagaagcccggccaggctcctagaggactgatcggcggaacaaacaaggaggccccttggacacccgccagattctctggatctctgctcggcggaaaggccgctctgacactttctggtgctcagcctgaggacgaggccgagtactattgtgccctgtggtacagcaacctgtgggtgttcggcggaggcaccaaactgacagttctg

SEQ ID NO: 18 - protein, 109 aa, Homo sapiens
QAVVTQEPSLTVSPGGTVTLTCRSSTGAVTTSNYANWVQEKPGQAPRGLIGGTNKRAPWTPARFSGSLLGGKAALTITGAQAEDEAEYYCVLWYSNLWVFGGGTKLTVL

SEQ ID NO: 19 - DNA, 327 bp, Homo sapiens
  source 1..327: mol_type = other DNA
caggctgtggtcacacaagagcctagcctgacagtgtctcctggcggcacagtgaccctgacctgtagatcttctacaggcgccgtgaccaccagcaactacgctaattgggtgcaggagaagcccggccaggctcctagaggactgatcggcggaacaaacaagagagccccttggacacccgccagattctctggatctctgctcggcggaaaggccgctctgacaatcactggtgctcaggctgaggacgaggccgagtactattgtgtgctgtggtacagcaacctgtgggtgttcggcggaggcaccaaactgacagttctg

SEQ ID NO: 20 - protein, 8 aa, Homo sapiens
YGTNKRAP

SEQ ID NO: 21 - protein, 9 aa, Homo sapiens
VLWYSNLWV

SEQ ID NO: 22 - protein, 109 aa, Homo sapiens
QAVVTQEPSLTVSPGGTVTLTCRSSTGAVTTSNYANWFQEKPGQAPRGLIYGTNKRAPWTPARFSGSLLGGKAALTLSGAQAEDEAEYYCVLWYSNLWVFGGGTKLTVL

SEQ ID NO: 23 - DNA, 327 bp, Homo sapiens
  source 1..327: mol_type = other DNA
caggctgtggtcacacaagagcctagcctgacagtgtctcctggcggcacagtgaccctgacctgtagatcttctacaggcgccgtgaccaccagcaactacgctaattggttccaggagaagcccggccaggctcctagaggactgatctacggaacaaacaagagagccccttggacacccgccagattctctggatctctgctcggcggaaaggccgctctgacactttctggtgctcaggctgaggacgaggccgagtactattgtgtcctgtggtacagcaacctgtgggtgttcggcggaggcaccaaactgacagttctg

SEQ ID NO: 24 - protein, 125 aa, Homo sapiens
EVQLVESGGGLVQPGGSLRLSCAASGFTFNTYAMNWVRQAPGKGLEWVSRIRSKYNNYATYYADSVKDRFTISRDDSKNTLYLQMNSLRAEDTAVYYCVRHGNFGNSYVSWFAYWGQGTLVTVSS

SEQ ID NO: 25 - DNA, 375 bp, Homo sapiens
  source 1..375: mol_type = other DNA
gaggtgcagctggttgaatctggcggaggactggttcagcctggcggatctctgagactgtcttgtgccgccagcggcttcaccttcaacacctacgctatgaactgggtccgacaggcccctggcaaaggactggaatgggtgtccagaatcaggtccaagtacaacaactacgccacctactacgccgacagcgtgaaggacagattcaccatcagcagggacgacagcaagaacaccctgtacctgcagatgaacagcctgagagccgaggacaccgccgtgtactactgtgtcagacacggcaacttcggcaacagctatgtgtcttggtttgcctactggggccagggcacactggtcacagttagctct

SEQ ID NO: 26 - protein, 6 aa, Homo sapiens
NTYAMN

SEQ ID NO: 27 - protein, 18 aa, Homo sapiens
IRSKYNNYATYYADSVKD

SEQ ID NO: 28 - protein, 14 aa, Homo sapiens
HGNFGNSYVSWFAY

SEQ ID NO: 29 - protein, 125 aa, Homo sapiens
EVQLVESGGGLVQPGGSLRLSCAASGFTFSTYAMNWVRKAPGKGLEWVSRIRSKYNNYATYYADSVKDRFTISRDDSKNTLYLQMNSLRAEDTAVYYCVRHGNFGNSYVSWFAYWGQGTLVTVSS

SEQ ID NO: 30 - DNA, 375 bp, Homo sapiens
  source 1..375: mol_type = other DNA
gaggtgcagctggttgaatctggcggaggactggttcagcctggcggatctctgagactgtcttgtgccgccagcggcttcaccttctccacctacgctatgaactgggtccgaaaggcccctggcaaaggactggaatgggtgtccagaatcaggtccaagtacaacaactacgccacctactacgccgacagcgtgaaggacagattcaccatcagcagggacgacagcaagaacaccctgtacctgcagatgaacagcctgagagccgaggacaccgccgtgtactactgtgtcagacacggcaacttcggcaacagctatgtgtcttggtttgcctactggggccagggcacactggtcacagttagctct

SEQ ID NO: 31 - protein, 6 aa, Homo sapiens
STYAMN

SEQ ID NO: 32 - protein, 125 aa, Homo sapiens
EVQLVESGGGLVQPGGSLRLSCAASGFTFSTYAMNWVRKAPGKGLEWVSRIRSKYNNYATYYADSVKDRFTISRDDSKNTLYLQMNSLRAEDTAVYYCVRHGNFGESYVSWFAYWGQGTLVTVSS

SEQ ID NO: 33 - DNA, 375 bp, Homo sapiens
  source 1..375: mol_type = other DNA
gaggtgcagctggttgaatctggcggaggactggttcagcctggcggatctctgagactgtcttgtgccgccagcggcttcaccttctccacctacgctatgaactgggtccgaaaggcccctggcaaaggactggaatgggtgtccagaatcaggtccaagtacaacaactacgccacctactacgccgacagcgtgaaggacagattcaccatcagcagggacgacagcaagaacaccctgtacctgcagatgaacagcctgagagccgaggacaccgccgtgtactactgtgtcagacacggcaacttcggcgagagctatgtgtcttggtttgcctactggggccagggcacactggtcacagttagctct

SEQ ID NO: 34 - protein, 14 aa, Homo sapiens
HGNFGESYVSWFAY

SEQ ID NO: 35 - protein, 125 aa, Homo sapiens
EVQLVESGGGLVQPGGSLRLSCAASGFTFSTYAMNWVRKAPGKGLEWVSRIRSKYNNYATYYADSVKDRFTISRDDSKNTLYLQMNSLRAEDTAVYYCVRHGNFGQSYVSWFAYWGQGTLVTVSS

SEQ ID NO: 36 - DNA, 375 bp, Homo sapiens
  source 1..375: mol_type = other DNA
gaggtgcagctggttgaatctggcggaggactggttcagcctggcggatctctgagactgtcttgtgccgccagcggcttcaccttctccacctacgctatgaactgggtccgaaaggcccctggcaaaggactggaatgggtgtccagaatcaggtccaagtacaacaactacgccacctactacgccgacagcgtgaaggacagattcaccatcagcagggacgacagcaagaacaccctgtacctgcagatgaacagcctgagagccgaggacaccgccgtgtactactgtgtcagacacggcaacttcggccagagctatgtgtcttggtttgcctactggggccagggcacactggtcacagttagctct

SEQ ID NO: 37 - protein, 14 aa, Homo sapiens
HGNFGQSYVSWFAY

SEQ ID NO: 38 - protein, 125 aa, Homo sapiens
EVQLVESGGGLVQPGGSLRLSCAASGFTFSTYAMNWVRKAPGKGLEWVSRIRSKYNNYATYYADSVKDRFTISRDDSKNTLYLQMNSLRAEDTAVYYCVRHGNFGDSYVSWFAYWGQGTLVTVSS

SEQ ID NO: 39 - DNA, 375 bp, Homo sapiens
  source 1..375: mol_type = other DNA
gaggtgcagctggttgaatctggcggaggactggttcagcctggcggatctctgagactgtcttgtgccgccagcggcttcaccttctccacctacgctatgaactgggtccgaaaggcccctggcaaaggactggaatgggtgtccagaatcaggtccaagtacaacaactacgccacctactacgccgacagcgtgaaggacagattcaccatcagcagggacgacagcaagaacaccctgtacctgcagatgaacagcctgagagccgaggacaccgccgtgtactactgtgtcagacacggcaacttcggcgacagctatgtgtcttggtttgcctactggggccagggcacactggtcacagttagctct

SEQ ID NO: 40 - protein, 14 aa, Homo sapiens
HGNFGDSYVSWFAY

SEQ ID NO: 41 - protein, 125 aa, Homo sapiens
EVQLVESGGGLVQPGGSLRLSCAASGFTFSTYAMNWVRKAPGKGLEWVSRIRSKYNNYATYYADSVKDRFTISRDDSKNTLYLQMNSLRAEDTAVYYCVRHGNFGTSYVSWFAYWGQGTLVTVSS

SEQ ID NO: 42 - DNA, 375 bp, Homo sapiens
  source 1..375: mol_type = other DNA
gaggtgcagctggttgaatctggcggaggactggttcagcctggcggatctctgagactgtcttgtgccgccagcggcttcaccttctccacctacgctatgaactgggtccgaaaggcccctggcaaaggactggaatgggtgtccagaatcaggtccaagtacaacaactacgccacctactacgccgacagcgtgaaggacagattcaccatcagcagggacgacagcaagaacaccctgtacctgcagatgaacagcctgagagccgaggacaccgccgtgtactactgtgtcagacacggcaacttcggcaccagctatgtgtcttggtttgcctactggggccagggcacactggtcacagttagctct

SEQ ID NO: 43 - protein, 14 aa, Homo sapiens
HGNFGTSYVSWFAY

SEQ ID NO: 44 - protein, 125 aa, Homo sapiens
EVQLVESGGGLVQPGGSLRLSCAASGFTFSDYAMNWVRKAPGKGLEWVSRIRSKYNNYATYYADSVEDRFTISRDDSKNTLYLQMNSLRAEDTAVYYCVRHGNFGNSYVSWFAYWGQGTLVTVSS

SEQ ID NO: 45 - DNA, 375 bp, Homo sapiens
  source 1..375: mol_type = other DNA
gaggtgcagctggttgaatctggcggaggactggttcagcctggcggatctctgagactgtcttgtgccgccagcggcttcaccttctccgactacgctatgaactgggtccgaaaggcccctggcaaaggactggaatgggtgtccagaatcaggtccaagtacaacaactacgccacctactacgccgacagcgtggaggacagattcaccatcagcagggacgacagcaagaacaccctgtacctgcagatgaacagcctgagagccgaggacaccgccgtgtactactgtgtcagacacggcaacttcggcaacagctatgtgtcttggtttgcctactggggccagggcacactggtcacagttagctct

SEQ ID NO: 46 - protein, 6 aa, Homo sapiens
SDYAMN

SEQ ID NO: 47 - protein, 18 aa, Homo sapiens
IRSKYNNYATYYADSVED

SEQ ID NO: 48 - protein, 125 aa, Homo sapiens
EVQLVESGGGLVQPGGSLRLSCAASGFTFNTYAMNWVRKAPGKGLEWVGRIRSKYNNYATYYADSVKDRFTISRDDSKNSLYLQMNSLKTEDTAVYYCARHGNFGNSYVSWFAYWGQGTLVTVSS

SEQ ID NO: 49 - DNA, 375 bp, Homo sapiens
  source 1..375: mol_type = other DNA
gaggtgcagctggttgaatctggcggaggactggttcagcctggcggatctctgagactgtcttgtgccgccagcggcttcaccttcaacacctacgctatgaactgggtccgaaaggcccctggcaaaggactggaatgggtgggaagaatcaggtccaagtacaacaactacgccacctactacgccgacagcgtgaaggacagattcaccatcagcagggacgacagcaagaacagcctgtacctgcagatgaacagcctgaaaaccgaggacaccgccgtgtactactgtgccagacacggcaacttcggcaacagctatgtgtcttggtttgcctactggggccagggcacactggtcacagttagctct

SEQ ID NO: 50 - protein, 125 aa, Homo sapiens
EVQLVESGGGLVQPGGSLRLSCAASGFTFNTYAMNWVRKAPGKGLEWVGRIRSKYNNYATYYADSVKDRFTISRDDSKNSLYLQMNSLKTEDTAVYYCVRHGNFGNSYVSWFAYWGQGTLVTVSS

SEQ ID NO: 51 - DNA, 375 bp, Homo sapiens
  source 1..375: mol_type = other DNA
gaggtgcagctggttgaatctggcggaggactggttcagcctggcggatctctgagactgtcttgtgccgccagcggcttcaccttcaacacctacgctatgaactgggtccgaaaggcccctggcaaaggactggaatgggtgggaagaatcaggtccaagtacaacaactacgccacctactacgccgacagcgtgaaggacagattcaccatcagcagggacgacagcaagaacagcctgtacctgcagatgaacagcctgaaaaccgaggacaccgccgtgtactactgtgtcagacacggcaacttcggcaacagctatgtgtcttggtttgcctactggggccagggcacactggtcacagttagctct

SEQ ID NO: 52 - protein, 125 aa, Homo sapiens
EVQLVESGGGLVQPGGSLRLSCAASGFTFNTYAMNWVRKAPGKGLEWVARIRSKYNNYATYYADSVKDRFTISRDDSKNSLYLQMNSLKTEDTAVYYCVRHGNFGNSYVSWFAYWGQGTLVTVSS

SEQ ID NO: 53 - DNA, 375 bp, Homo sapiens
  source 1..375: mol_type = other DNA
gaggtgcagctggttgaatctggcggaggactggttcagcctggcggatctctgagactgtcttgtgccgccagcggcttcaccttcaacacctacgctatgaactgggtccgaaaggcccctggcaaaggactggaatgggtggccagaatcaggtccaagtacaacaactacgccacctactacgccgacagcgtgaaggacagattcaccatcagcagggacgacagcaagaacagcctgtacctgcagatgaacagcctgaaaaccgaggacaccgccgtgtactactgtgtcagacacggcaacttcggcaacagctatgtgtcttggtttgcctactggggccagggcacactggtcacagttagctct

SEQ ID NO: 54 - protein, 214 aa, Homo sapiens
EIVLTQSPGTLSLSPGERATLSCRASQSVSSYLAWYQQKPGQAPRLLIYDASNRATGIPDRFSGSGSGTDFTLTISRLEPEDFAVYYCQQRSNWPITFGQGTKLEIKRTVAAPSVFIFPPSDEQLKSGTASVVCLLNNFYPREAKVQWKVDNALQSGNSQESVTEQDSKDSTYSLSSTLTLSKADYEKHKVYACEVTHQGLSSPVTKSFNRGEC

SEQ ID NO: 55 - DNA, 642 bp, Homo sapiens
  source 1..642: mol_type = other DNA
gagatcgtgctgacacagagccctggcacactgtcactgtctccaggcgagagagccacactgagctgtagagccagccagagcgtgtcctcttacctggcctggtatcagcagaagcctggacaggctcccagactgctgatctacgacgccagcaacagagccacaggcatccccgatagattcagcggctctggctctggcaccgacttcaccctgacaatcagcagactggaacccgaggacttcgccgtgtactactgccagcagagaagcaactggcccatcacattcggccagggcaccaagctggaaatcaagcgaactgtggctgcaccatctgtcttcatcttcccgccatctgatgagcagttgaaatctggaactgcctctgttgtgtgcctgctgaataacttctatcccagagaggccaaagtacagtggaaggtggataacgccctccaatcgggtaactcccaggagagtgtcacagagcaggacagcaaggacagcacctacagcctcagcagcaccctgacgctgagcaaagcagactacgagaaacacaaagtctacgcctgcgaagtcacccatcagggcctgagctcgcccgtcacaaagagcttcaacaggggagagtgt

SEQ ID NO: 56 - protein, 449 aa, Homo sapiens
EVQLLESGGGVVQPGGSLRLSCAASGFTFNDYAMHWVRQAPGKGLEWVSTISWNSGSIGYADSVKGRFTISRDNSKNTLYLQMNSLRAEDTAVYYCAKDIQYGNYYYGMDYWGQGTLVTVSSASTKGPSVFPLAPCSRSTSESTAALGCLVKDYFPEPVTVSWNSGALTSGVHTFPAVLQSSGLYSLSSVVTVPSSSLGTKTYTCNVDHKPSNTKVDKRVESKYGPPCPPCPAPEFEGGPSVFLFPPKPKDTLMISRTPEVTCVVVDVSQEDPEVQFNWYVDGVEVHNAKTKPREEQFNSTYRVVSVLTVLHQDWLNGKEYKCKVSNKGLASSIEKTISKAKGQPREPQVCTLPPSQEEMTKNQVSLSCAVKGFYPSDIAVEWESNGQPENNYKTTPPVLDSDGSFFLVSKLTVDKSRWQEGNVFSCSVMHEALHNHYTQKSLSLSLGK

SEQ ID NO: 57 - DNA, 1347 bp, Homo sapiens
  source 1..1347: mol_type = other DNA
gaagtgcagctgctggaatctggtggcggagttgttcagcctggcggctctctgagactgtcttgtgctgccagcggcttcaccttcaacgactacgctatgcactgggtccgacaggcccctggcaaaggacttgaatgggtgtccaccatcagctggaacagcggctctatcggctacgccgattccgtgaagggcagattcaccatctccagagacaacagcaagaacaccctgtacctgcagatgaacagcctgagagccgaggacaccgccgtgtactactgtgccaaggacatccagtacggcaactactactacggcatggactactggggccagggaacactggttaccgttagctctgctagcaccaagggccccagcgtgttccccctggccccttgcagcagaagcaccagcgagagcacagccgccctgggctgcctggtgaaggactacttccccgagcccgtgaccgtgtcctggaacagcggcgctctgaccagcggcgtgcataccttccccgccgtgctccagagcagcggactgtactccctgagcagcgtggtgaccgtgccttccagcagcctgggcaccaagacctacacctgcaacgtggaccacaagcccagcaacaccaaggtggacaagagagtggagagcaagtacggccctccctgccccccttgccctgcccccgagttcgagggcggacctagcgtgttcctgttcccccccaagcccaaggacaccctgatgatcagcagaacccccgaggtgacctgcgtggtggtggacgtgtcccaggaggaccccgaggtccagtttaattggtacgtggacggcgtggaagtgcataacgccaagaccaagcccagagaggagcagttcaacagcacctacagagtggtgtccgtgctgaccgtgctgcaccaggactggctgaacggcaaggaatacaagtgcaaggtctccaacaagggcctggccagcagcatcgagaagaccatcagcaaggccaagggccagccacgggagccccaggtctgcaccctgccacctagccaagaggagatgaccaagaaccaggtgtccctgagctgtgccgtgaaaggcttctatcccagcgatatcgccgtggagtgggagagcaacggccagcccgagaacaactacaagaccaccccccctgtgctggacagcgacggcagcttcttcctggtttccaagctgaccgtggacaagtccagatggcaggagggcaacgtcttcagctgctccgtgatgcacgaggccctgcacaaccactacacccagaagtccctgagcctgagcctgggcaag

SEQ ID NO: 58 - protein, 215 aa, Homo sapiens
QAVVTQEPSLTVSPGGTVTLTCRSSTGAVTTSNYANWVQQKPGQAPRGLIGGTNKRAPWTPARFSGSLLGGKAALTITGAQAEDEAEYYCVLWYSNLWVFGGGTKLTVLGQPKAAPSVTLFPPSSEELQANKATLVCLISDFYPGAVTVAWKADSSPVKAGVETTTPSKQSNNKYAASSYLSLTPEQWKSHRSYSCQVTHEGSTVEKTVAPTECS

SEQ ID NO: 59 - DNA, 645 bp, Homo sapiens
  source 1..645: mol_type = other DNA
caggctgtggtcacacaagagcctagcctgacagtgtctcctggcggcacagtgaccctgacctgtagatcttctacaggcgccgtgaccaccagcaactacgctaattgggtgcagcagaagcccggccaggctcctagaggactgatcggcggaacaaacaagagagccccttggacacccgccagattctctggatctctgctcggcggaaaggccgctctgacaatcactggtgctcaggctgaggacgaggccgagtactattgtgtgctgtggtacagcaacctgtgggtgttcggcggaggcaccaaactgacagttctgggtcagcccaaggcggcgccctcggtcactctgttcccgccctcctctgaggagcttcaagccaacaaggccacactggtgtgtctcataagtgacttctatccgggagccgtgacagtggcctggaaggcagatagcagccccgtcaaggcgggagtggagaccaccacaccctccaaacaaagcaacaacaagtacgcggccagcagctacctgagcctgacgcctgagcagtggaagtcccacagaagctacagctgccaggtcacgcatgaagggagcaccgtggagaagacagtggcccctacagaatgttca

SEQ ID NO: 60 - protein, 452 aa, Homo sapiens
EVQLVESGGGLVQPGGSLRLSCAASGFTFNTYAMNWVRQAPGKGLEWVGRIRSKYNNYATYYADSVKDRFTISRDDSKNSLYLQMNSLKTEDTAVYYCVRHGNFGNSYVSWFAYWGQGTLVTVSSASTKGPSVFPLAPCSRSTSESTAALGCLVKDYFPEPVTVSWNSGALTSGVHTFPAVLQSSGLYSLSSVVTVPSSSLGTKTYTCNVDHKPSNTKVDKRVESKYGPPCPPCPAPEFEGGPSVFLFPPKPKDTLMISRTPEVTCVVVDVSQEDPEVQFNWYVDGVEVHNAKTKPREEQFNSTYRVVSVLTVLHQDWLNGKEYKCKVSNKGLASSIEKTISKAKGQPREPQVYTLPPCQEEMTKNQVSLWCLVKGFYPSDIAVEWESNGQPENNYKTTPPVLDSDGSFFLYSKLTVDKSRWQEGNVFSCSVMHEALHNHYTQKSLSLSLGK

SEQ ID NO: 61 - DNA, 1356 bp, Homo sapiens
  source 1..1356: mol_type = other DNA
gaggtgcagctggttgaatctggcggaggactggttcagcctggcggatctctgagactgtcttgtgccgccagcggcttcaccttcaacacctacgctatgaactgggtccgacaggcccctggcaaaggactggaatgggtgggaagaatcaggtccaagtacaacaactacgccacctactacgccgacagcgtgaaggacagattcaccatcagcagggacgacagcaagaacagcctgtacctgcagatgaacagcctgaaaaccgaggacaccgccgtgtactactgtgtcagacacggcaacttcggcaacagctatgtgtcttggtttgcctactggggccagggcacactggtcacagttagctctgctagcaccaagggccccagcgtgttccccctggccccttgcagcagaagcaccagcgagagcacagccgccctgggctgcctggtgaaggactacttccccgagcccgtgaccgtgtcctggaacagcggcgctctgaccagcggcgtgcataccttccccgccgtgctccagagcagcggactgtactccctgagcagcgtggtgaccgtgccttccagcagcctgggcaccaagacctacacctgcaacgtggaccacaagcccagcaacaccaaggtggacaagagagtggagagcaagtacggccctccctgccccccttgccctgcccccgagttcgagggcggacctagcgtgttcctgttcccccccaagcccaaggacaccctgatgatcagcagaacccccgaggtgacctgcgtggtggtggacgtgtcccaggaggaccccgaggtccagtttaattggtacgtggacggcgtggaagtgcataacgccaagaccaagcccagagaggagcagttcaacagcacctacagagtggtgtccgtgctgaccgtgctgcaccaggactggctgaacggcaaggaatacaagtgcaaggtctccaacaagggcctggccagcagcatcgagaagaccatcagcaaggccaagggccagccacgggagccccaggtctacaccctgccaccttgtcaagaggagatgaccaagaaccaggtgtccctgtggtgtctggtgaaaggcttctatcccagcgatatcgccgtggagtgggagagcaacggccagcccgagaacaactacaagaccaccccccctgtgctggacagcgacggcagcttcttcctgtactccaagctgaccgtggacaagtccagatggcaggagggcaacgtcttcagctgctccgtgatgcacgaggccctgcacaaccactacacccagaagtccctgagcctgagcctgggcaag

SEQ ID NO: 62 - protein, 214 aa, Homo sapiens
EIVLTQSPGTLSLSPGERATLSCRASQSVSSYLAWYQKKPGQAPRLLIYDASNRATGIPDRFSGSGSGTDFTLTISRLEPEDFAVYYCQQRSNWPITFGQGTKLEIKRTVAAPSVFIFPPSDEQLKSGTASVVCLLNNFYPREAKVQWKVDNALQSGNSQESVTEQDSKDSTYSLSSTLTLSKADYEKHKVYACEVTHQGLSSPVTKSFNRGEC

SEQ ID NO: 63 - DNA, 642 bp, Homo sapiens
  source 1..642: mol_type = other DNA
gagatcgtgctgacacagagccctggcacactgtcactgtctccaggcgagagagccacactgagctgtagagccagccagagcgtgtcctcttacctggcctggtatcagaagaagcctggacaggctcccagactgctgatctacgacgccagcaacagagccacaggcatccccgatagattcagcggctctggctctggcaccgacttcaccctgacaatcagcagactggaacccgaggacttcgccgtgtactactgccagcagagaagcaactggcccatcacattcggccagggcaccaagctggaaatcaagcgaactgtggctgcaccatctgtcttcatcttcccgccatctgatgagcagttgaaatctggaactgcctctgttgtgtgcctgctgaataacttctatcccagagaggccaaagtacagtggaaggtggataacgccctccaatcgggtaactcccaggagagtgtcacagagcaggacagcaaggacagcacctacagcctcagcagcaccctgacgctgagcaaagcagactacgagaaacacaaagtctacgcctgcgaagtcacccatcagggcctgagctcgcccgtcacaaagagcttcaacaggggagagtgt

SEQ ID NO: 64 - protein, 449 aa, Homo sapiens
EVQLLESGGGVVQPGGSLRLSCAASGFTFNDYAMHWVREAPGKGLEWVSTISWNSGSIGYADSVKGRFTISRDNSKNTLYLQMNSLRAEDTAVYYCAKDIQYGNYYYGMDYWGQGTLVTVSSASTKGPSVFPLAPCSRSTSESTAALGCLVKDYFPEPVTVSWNSGALTSGVHTFPAVLQSSGLYSLSSVVTVPSSSLGTKTYTCNVDHKPSNTKVDKRVESKYGPPCPPCPAPEFEGGPSVFLFPPKPKDTLMISRTPEVTCVVVDVSQEDPEVQFNWYVDGVEVHNAKTKPREEQFNSTYRVVSVLTVLHQDWLNGKEYKCKVSNKGLASSIEKTISKAKGQPREPQVCTLPPSQEEMTKNQVSLSCAVKGFYPSDIAVEWESNGQPENNYKTTPPVLDSDGSFFLVSKLTVDKSRWQEGNVFSCSVMHEALHNHYTQKSLSLSLGK

SEQ ID NO: 65 - DNA, 1347 bp, Homo sapiens
  source 1..1347: mol_type = other DNA
gaagtgcagctgctggaatctggtggcggagttgttcagcctggcggctctctgagactgtcttgtgctgccagcggcttcaccttcaacgactacgctatgcactgggtccgagaggcccctggcaaaggacttgaatgggtgtccaccatcagctggaacagcggctctatcggctacgccgattccgtgaagggcagattcaccatctccagagacaacagcaagaacaccctgtacctgcagatgaacagcctgagagccgaggacaccgccgtgtactactgtgccaaggacatccagtacggcaactactactacggcatggactactggggccagggaacactggttaccgttagctctgctagcaccaagggccccagcgtgttccccctggccccttgcagcagaagcaccagcgagagcacagccgccctgggctgcctggtgaaggactacttccccgagcccgtgaccgtgtcctggaacagcggcgctctgaccagcggcgtgcataccttccccgccgtgctccagagcagcggactgtactccctgagcagcgtggtgaccgtgccttccagcagcctgggcaccaagacctacacctgcaacgtggaccacaagcccagcaacaccaaggtggacaagagagtggagagcaagtacggccctccctgccccccttgccctgcccccgagttcgagggcggacctagcgtgttcctgttcccccccaagcccaaggacaccctgatgatcagcagaacccccgaggtgacctgcgtggtggtggacgtgtcccaggaggaccccgaggtccagtttaattggtacgtggacggcgtggaagtgcataacgccaagaccaagcccagagaggagcagttcaacagcacctacagagtggtgtccgtgctgaccgtgctgcaccaggactggctgaacggcaaggaatacaagtgcaaggtctccaacaagggcctggccagcagcatcgagaagaccatcagcaaggccaagggccagccacgggagccccaggtctgcaccctgccacctagccaagaggagatgaccaagaaccaggtgtccctgagctgtgccgtgaaaggcttctatcccagcgatatcgccgtggagtgggagagcaacggccagcccgagaacaactacaagaccaccccccctgtgctggacagcgacggcagcttcttcctggtttccaagctgaccgtggacaagtccagatggcaggagggcaacgtcttcagctgctccgtgatgcacgaggccctgcacaaccactacacccagaagtccctgagcctgagcctgggcaag

SEQ ID NO: 66 - protein, 215 aa, Homo sapiens
QAVVTQEPSLTVSPGGTVTLTCRSSTGAVTTSNYANWVQEKPGQAPRGLIGGTNKRAPWTPARFSGSLLGGKAALTITGAQAEDEAEYYCVLWYSNLWVFGGGTKLTVLGQPKAAPSVTLFPPSSEELQANKATLVCLISDFYPGAVTVAWKADSSPVKAGVETTTPSKQSNNKYAASSYLSLTPEQWKSHRSYSCQVTHEGSTVEKTVAPTECS

SEQ ID NO: 67 - DNA, 645 bp, Homo sapiens
  source 1..645: mol_type = other DNA
caggctgtggtcacacaagagcctagcctgacagtgtctcctggcggcacagtgaccctgacctgtagatcttctacaggcgccgtgaccaccagcaactacgctaattgggtgcaggagaagcccggccaggctcctagaggactgatcggcggaacaaacaagagagccccttggacacccgccagattctctggatctctgctcggcggaaaggccgctctgacaatcactggtgctcaggctgaggacgaggccgagtactattgtgtgctgtggtacagcaacctgtgggtgttcggcggaggcaccaaactgacagttctgggtcagcccaaggcggcgccctcggtcactctgttcccgccctcctctgaggagcttcaagccaacaaggccacactggtgtgtctcataagtgacttctatccgggagccgtgacagtggcctggaaggcagatagcagccccgtcaaggcgggagtggagaccaccacaccctccaaacaaagcaacaacaagtacgcggccagcagctacctgagcctgacgcctgagcagtggaagtcccacagaagctacagctgccaggtcacgcatgaagggagcaccgtggagaagacagtggcccctacagaatgttca

SEQ ID NO: 68 - protein, 452 aa, Homo sapiens
EVQLVESGGGLVQPGGSLRLSCAASGFTFNTYAMNWVRKAPGKGLEWVGRIRSKYNNYATYYADSVKDRFTISRDDSKNSLYLQMNSLKTEDTAVYYCVRHGNFGNSYVSWFAYWGQGTLVTVSSASTKGPSVFPLAPCSRSTSESTAALGCLVKDYFPEPVTVSWNSGALTSGVHTFPAVLQSSGLYSLSSVVTVPSSSLGTKTYTCNVDHKPSNTKVDKRVESKYGPPCPPCPAPEFEGGPSVFLFPPKPKDTLMISRTPEVTCVVVDVSQEDPEVQFNWYVDGVEVHNAKTKPREEQFNSTYRVVSVLTVLHQDWLNGKEYKCKVSNKGLASSIEKTISKAKGQPREPQVYTLPPCQEEMTKNQVSLWCLVKGFYPSDIAVEWESNGQPENNYKTTPPVLDSDGSFFLYSKLTVDKSRWQEGNVFSCSVMHEALHNHYTQKSLSLSLGK

SEQ ID NO: 69 - DNA, 1356 bp, Homo sapiens
  source 1..1356: mol_type = other DNA
gaggtgcagctggttgaatctggcggaggactggttcagcctggcggatctctgagactgtcttgtgccgccagcggcttcaccttcaacacctacgctatgaactgggtccgaaaggcccctggcaaaggactggaatgggtgggaagaatcaggtccaagtacaacaactacgccacctactacgccgacagcgtgaaggacagattcaccatcagcagggacgacagcaagaacagcctgtacctgcagatgaacagcctgaaaaccgaggacaccgccgtgtactactgtgtcagacacggcaacttcggcaacagctatgtgtcttggtttgcctactggggccagggcacactggtcacagttagctctgctagcaccaagggccccagcgtgttccccctggccccttgcagcagaagcaccagcgagagcacagccgccctgggctgcctggtgaaggactacttccccgagcccgtgaccgtgtcctggaacagcggcgctctgaccagcggcgtgcataccttccccgccgtgctccagagcagcggactgtactccctgagcagcgtggtgaccgtgccttccagcagcctgggcaccaagacctacacctgcaacgtggaccacaagcccagcaacaccaaggtggacaagagagtggagagcaagtacggccctccctgccccccttgccctgcccccgagttcgagggcggacctagcgtgttcctgttcccccccaagcccaaggacaccctgatgatcagcagaacccccgaggtgacctgcgtggtggtggacgtgtcccaggaggaccccgaggtccagtttaattggtacgtggacggcgtggaagtgcataacgccaagaccaagcccagagaggagcagttcaacagcacctacagagtggtgtccgtgctgaccgtgctgcaccaggactggctgaacggcaaggaatacaagtgcaaggtctccaacaagggcctggccagcagcatcgagaagaccatcagcaaggccaagggccagccacgggagccccaggtctacaccctgccaccttgtcaagaggagatgaccaagaaccaggtgtccctgtggtgtctggtgaaaggcttctatcccagcgatatcgccgtggagtgggagagcaacggccagcccgagaacaactacaagaccaccccccctgtgctggacagcgacggcagcttcttcctgtactccaagctgaccgtggacaagtccagatggcaggagggcaacgtcttcagctgctccgtgatgcacgaggccctgcacaaccactacacccagaagtccctgagcctgagcctgggcaag

SEQ ID NO: 70 - protein, 214 aa, Homo sapiens
EIVLTQSPGTLSLSPGERATLSCRASQSVSSYLAWYQKKPGQAPRLLIYDASNRATGIPDRFSGSGSGTDFTLTISRLEPEDFAVYYCQQRSNWPITFGQGTKLEIKRTVAAPSVFIFPPSDKKLKSGTASVVCLLNNFYPREAKVQWKVDNALQSGNSQESVTEQDSKDSTYSLSSTLTLSKADYEKHKVYACEVTHQGLSSPVTKSFNRGEC

SEQ ID NO: 71 - DNA, 642 bp, Homo sapiens
  source 1..642: mol_type = other DNA
gagatcgtgctgacacagagccctggcacactgtcactgtctccaggcgagagagccacactgagctgtagagccagccagagcgtgtcctcttacctggcctggtatcagaagaagcctggacaggctcccagactgctgatctacgacgccagcaacagagccacaggcatccccgatagattcagcggctctggctctggcaccgacttcaccctgacaatcagcagactggaacccgaggacttcgccgtgtactactgccagcagagaagcaactggcccatcacattcggccagggcaccaagctggaaatcaagcgaactgtggctgcaccatctgtcttcatcttcccgccatctgataagaaattgaaatctggaactgcctctgttgtgtgcctgctgaataacttctatcccagagaggccaaagtacagtggaaggtggataacgccctccaatcgggtaactcccaggagagtgtcacagagcaggacagcaaggacagcacctacagcctcagcagcaccctgacgctgagcaaagcagactacgagaaacacaaagtctacgcctgcgaagtcacccatcagggcctgagctcgcccgtcacaaagagcttcaacaggggagagtgt

SEQ ID NO: 72 - protein, 449 aa, Homo sapiens
EVQLLESGGGVVQPGGSLRLSCAASGFTFNDYAMHWVREAPGKGLEWVSTISWNSGSIGYADSVKGRFTISRDNSKNTLYLQMNSLRAEDTAVYYCAKDIQYGNYYYGMDYWGQGTLVTVSSASTKGPSVFPLAPCSRSTSESTAALGCLVEDYFPEPVTVSWNSGALTSGVHTFPAVLQSSGLYSLSSVVTVPSSSLGTKTYTCNVDHKPSNTKVDERVESKYGPPCPPCPAPEFEGGPSVFLFPPKPKDTLMISRTPEVTCVVVDVSQEDPEVQFNWYVDGVEVHNAKTKPREEQFNSTYRVVSVLTVLHQDWLNGKEYKCKVSNKGLASSIEKTISKAKGQPREPQVCTLPPSQEEMTKNQVSLSCAVKGFYPSDIAVEWESNGQPENNYKTTPPVLDSDGSFFLVSKLTVDKSRWQEGNVFSCSVMHEALHNHYTQKSLSLSLGK

SEQ ID NO: 73 - DNA, 1347 bp, Homo sapiens
  source 1..1347: mol_type = other DNA
gaagtgcagctgctggaatctggtggcggagttgttcagcctggcggctctctgagactgtcttgtgctgccagcggcttcaccttcaacgactacgctatgcactgggtccgagaggcccctggcaaaggacttgaatgggtgtccaccatcagctggaacagcggctctatcggctacgccgattccgtgaagggcagattcaccatctccagagacaacagcaagaacaccctgtacctgcagatgaacagcctgagagccgaggacaccgccgtgtactactgtgccaaggacatccagtacggcaactactactacggcatggactactggggccagggaacactggttaccgttagctctgctagcaccaagggccccagcgtgttccccctggccccttgcagcagaagcaccagcgagagcacagccgccctgggctgcctggtggaggactacttccccgagcccgtgaccgtgtcctggaacagcggcgctctgaccagcggcgtgcataccttccccgccgtgctccagagcagcggactgtactccctgagcagcgtggtgaccgtgccttccagcagcctgggcaccaagacctacacctgcaacgtggaccacaagcccagcaacaccaaggtggacgagagagtggagagcaagtacggccctccctgccccccttgccctgcccccgagttcgaaggcggacctagcgtgttcctgttcccccccaagcccaaggacaccctgatgatcagcagaacccccgaggtgacctgcgtggtggtggacgtgtcccaggaggaccccgaggtccagtttaattggtacgtggacggcgtggaagtgcataacgccaagaccaagcccagagaggagcagttcaacagcacctacagagtggtgtccgtgctgaccgtgctgcaccaggactggctgaacggcaaggaatacaagtgcaaggtctccaacaagggcctggccagcagcatcgagaagaccatcagcaaggccaagggccagccacgggagccccaggtctgcaccctgccacctagccaagaggagatgaccaagaaccaggtgtccctgagctgtgccgtgaaaggcttctatcccagcgatatcgccgtggagtgggagagcaacggccagcccgagaacaactacaagaccaccccccctgtgctggacagcgacggcagcttcttcctggtttccaagctgaccgtggacaagtccagatggcaggagggcaacgtcttcagctgctccgtgatgcacgaggccctgcacaaccactacacccagaagtccctgagcctgagcctgggcaag

SEQ ID NO: 74 - protein, 449 aa, Homo sapiens
EVQLLESGGGVVQPGGSLRLSCAASGFTFNDYAMHWVREAPGKGLEWVSTISWNSGSIGYADSVKGRFTISRDNSKNTLYLQMNSLRAEDTAVYYCAKDIQYGNYYYGMDYWGQGTLVTVSSASTKGPSVFPLAPCSRSTSESTAALGCLVEDYFPEPVTVSWNSGALTSGVHTFPAVLQSSGLYSLSSVVTVPSSSLGTKTYTCNVDHKPSNTKVDERVESKYGPPCPPCPAPEFEGGPSVFLFPPKPKDTLMISRTPEVTCVVVDVSQEDPEVQFNWYVDGVEVHNAKTKPREEQFASTYRVVSVLTVLHQDWLNGKEYKCKVSNKGLPSSIEKTISKAKGQPREPQVCTLPPSQEEMTKNQVSLSCAVKGFYPSDIAVEWESNGQPENNYKTTPPVLDSDGSFFLVSKLTVDKSRWQEGNVFSCSVMHEALHNHYTQKSLSLSLGK

SEQ ID NO: 75 - DNA, 1347 bp, Homo sapiens
  source 1..1347: mol_type = other DNA
gaagtgcagctgctggaatctggtggcggagttgttcagcctggcggctctctgagactgtcttgtgctgccagcggcttcaccttcaacgactacgctatgcactgggtccgagaggcccctggcaaaggacttgaatgggtgtccaccatcagctggaacagcggctctatcggctacgccgattccgtgaagggcagattcaccatctccagagacaacagcaagaacaccctgtacctgcagatgaacagcctgagagccgaggacaccgccgtgtactactgtgccaaggacatccagtacggcaactactactacggcatggactactggggccagggaacactggttaccgttagctctgctagcaccaagggccccagcgtgttccccctggccccttgcagcagaagcaccagcgagagcacagccgccctgggctgcctggtggaggactacttccccgagcccgtgaccgtgtcctggaacagcggcgctctgaccagcggcgtgcataccttccccgccgtgctccagagcagcggactgtactccctgagcagcgtggtgaccgtgccttccagcagcctgggcaccaagacctacacctgcaacgtggaccacaagcccagcaacaccaaggtggacgagagagtggagagcaagtacggccctccctgccccccttgccctgcccccgagttcgaaggcggacctagcgtgttcctgttcccccccaagcccaaggacaccctgatgatcagcagaacccccgaggtgacctgcgtggtggtggacgtgtcccaggaggaccccgaggtccagtttaattggtacgtggacggcgtggaagtgcataacgccaagaccaagcccagagaggagcagttcgccagcacctacagagtggtgtccgtgctgaccgtgctgcaccaggactggctgaacggcaaggaatacaagtgcaaggtctccaacaagggcctgcctagcagcatcgagaagaccatcagcaaggccaagggccagccacgggagccccaggtctgcaccctgccacctagccaagaggagatgaccaagaaccaggtgtccctgagctgtgccgtgaaaggcttctatcccagcgatatcgccgtggagtgggagagcaacggccagcccgagaacaactacaagaccaccccccctgtgctggacagcgacggcagcttcttcctggtttccaagctgaccgtggacaagtccagatggcaggagggcaacgtcttcagctgctccgtgatgcacgaggccctgcacaaccactacacccagaagtccctgagcctgagcctgggcaag

SEQ ID NO: 76 - protein, 223 aa, Homo sapiens
EVQLVESGGGLVQPGGSLRLSCAASGFTFNTYAMNWVRKAPGKGLEWVGRIRSKYNNYATYYADSVKDRFTISRDDSKNSLYLQMNSLKTEDTAVYYCVRHGNFGNSYVSWFAYWGQGTLVTVSSASTKGPSVFPLAPCSRSTSESTAALGCLVKDYFPEPVTVSWNSGALTSGVHTFPAVLQSSGLYSLSSVVTVPSSSLGTKTYTCNVDHKPSNTKVDKRV

SEQ ID NO: 77 - DNA, 669 bp, Homo sapiens
  source 1..669: mol_type = other DNA
gaggtgcagctggttgaatctggcggaggactggttcagcctggcggatctctgagactgtcttgtgccgccagcggcttcaccttcaacacctacgctatgaactgggtccgaaaggcccctggcaaaggactggaatgggtgggaagaatcaggtccaagtacaacaactacgccacctactacgccgacagcgtgaaggacagattcaccatcagcagggacgacagcaagaacagcctgtacctgcagatgaacagcctgaaaaccgaggacaccgccgtgtactactgtgtcagacacggcaacttcggcaacagctatgtgtcttggtttgcctactggggccagggcacactggtcacagttagctctgctagcaccaagggccccagcgtgttccccctggccccttgcagcagaagcaccagcgagagcacagccgccctgggctgcctggtgaaggactacttccccgagcccgtgaccgtgtcctggaacagcggcgctctgaccagcggcgtgcataccttccccgccgtgctccagagcagcggactgtactccctgagcagcgtggtgaccgtgccttccagcagcctgggcaccaagacctacacctgcaacgtggaccacaagcccagcaacaccaaggtggacaagagagtg

SEQ ID NO: 78 - protein, 444 aa, Homo sapiens
QAVVTQEPSLTVSPGGTVTLTCRSSTGAVTTSNYANWVQEKPGQAPRGLIGGTNKRAPWTPARFSGSLLGGKAALTITGAQAEDEAEYYCVLWYSNLWVFGGGTKLTVLGQPKAAPSVTLFPPSSEELQANKATLVCLISDFYPGAVTVAWKADSSPVKAGVETTTPSKQSNNKYAASSYLSLTPEQWKSHRSYSCQVTHEGSTVEKTVAPTECSESKYGPPCPPCPAPEFEGGPSVFLFPPKPKDTLMISRTPEVTCVVVDVSQEDPEVQFNWYVDGVEVHNAKTKPREEQFASTYRVVSVLTVLHQDWLNGKEYKCKVSNKGLPSSIEKTISKAKGQPREPQVYTLPPCQEEMTKNQVSLWCLVKGFYPSDIAVEWESNGQPENNYKTTPPVLDSDGSFFLYSKLTVDKSRWQEGNVFSCSVMHEALHNHYTQKSLSLSLGK

SEQ ID NO: 79 - DNA, 1332 bp, Homo sapiens
  source 1..1332: mol_type = other DNA
caggctgtggtcacacaagagcctagcctgacagtgtctcctggcggcacagtgaccctgacctgtagatcttctacaggcgccgtgaccaccagcaactacgctaattgggtgcaggagaagcccggccaggctcctagaggactgatcggcggaacaaacaagagagccccttggacacccgccagattctctggatctctgctcggcggaaaggccgctctgacaatcactggtgctcaggctgaggacgaggccgagtactattgtgtgctgtggtacagcaacctgtgggtgttcggcggaggcaccaaactgacagttctgggtcagcccaaggcggcgccctcggtcactctgttcccgccctcctctgaggagcttcaagccaacaaggccacactggtgtgtctcataagtgacttctatccgggagccgtgacagtggcctggaaggcagatagcagccccgtcaaggcgggagtggagaccaccacaccctccaaacaaagcaacaacaagtacgcggccagcagctacctgagcctgacgcctgagcagtggaagtcccacagaagctacagctgccaggtcacgcatgaagggagcaccgtggagaagacagtggcccctacagaatgttcagagagcaagtacggccctccctgccccccttgccctgcccccgagttcgagggcggacctagcgtgttcctgttcccccccaagcccaaggacaccctgatgatcagcagaacccccgaggtgacctgcgtggtggtggacgtgtcccaggaggaccccgaggtccagtttaattggtacgtggacggcgtggaagtgcataacgccaagaccaagcccagagaggagcagttcgccagcacctacagagtggtgtccgtgctgaccgtgctgcaccaggactggctgaacggcaaggaatacaagtgcaaggtctccaacaagggcctgcctagcagcatcgagaagaccatcagcaaggccaagggccagccacgggagccccaggtctacaccctgccaccttgtcaagaggagatgaccaagaaccaggtgtccctgtggtgtctggtgaaaggcttctatcccagcgatatcgccgtggagtgggagagcaacggccagcccgagaacaactacaagaccaccccccctgtgctggacagcgacggcagcttcttcctgtactccaagctgaccgtggacaagtccagatggcaggagggcaacgtcttcagctgctccgtgatgcacgaggccctgcacaaccactacacccagaagtccctgagcctgagcctgggcaag

SEQ ID NO: 80 - protein, 218 aa, Homo sapiens
DIVLTQSPASLAVSPGQRATITCRASKSVSTSGYSYMHWYQKKPGQPPKLLIYLASNLESGVPARFSGSGSGTDFTLTINPVEAEDTANYYCQHSRELPWTFGQGTKVEIKRTVAAPSVFIFPPSDEQLKSGTASVVCLLNNFYPREAKVQWKVDNALQSGNSQESVTEQDSKDSTYSLSSTLTLSKADYEKHKVYACEVTHQGLSSPVTKSFNRGEC

SEQ ID NO: 81 - DNA, 654 bp, Homo sapiens
  source 1..654: mol_type = other DNA
gacatcgtgctgacacagagccctgcttctctggctgtgtctcctggccagagagccaccatcacctgtagagccagcaagagcgtgtccaccagcggctactcttacatgcactggtatcagaagaagcccggccagcctcctaagctgctgatctacctggctagcaacctcgaaagcggagtgcctgctagattttctggcagcggctctggcaccgacttcaccctgacaatcaaccccgtggaagccgaagacaccgccaactactactgccagcacagcagagagctgccctggacatttggccagggcaccaaggtggaaatcaagcgaactgtggctgcaccatctgtcttcatcttcccgccatctgatgagcagttgaaatctggaactgcctctgttgtgtgcctgctgaataacttctatcccagagaggccaaagtacagtggaaggtggataacgccctccaatcgggtaactcccaggagagtgtcacagagcaggacagcaaggacagcacctacagcctcagcagcaccctgacgctgagcaaagcagactacgagaaacacaaagtctacgcctgcgaagtcacccatcagggcctgagctcgcccgtcacaaagagcttcaacaggggagagtgt

SEQ ID NO: 82 - protein, 449 aa, Homo sapiens
QVQLVQSGSELKKPGASVKVSCKASGYIFTNFGMNWVREAPGQGLEWMGWINTYTGEQIYADGFTGRFVFSLDTSASTAYLQISSLKAEDTAVYFCARGEIYYGYDVGFVYWGQGTLVTVSSASTKGPSVFPLAPCSRSTSESTAALGCLVKDYFPEPVTVSWNSGALTSGVHTFPAVLQSSGLYSLSSVVTVPSSSLGTKTYTCNVDHKPSNTKVDKRVESKYGPPCPPCPAPEFEGGPSVFLFPPKPKDTLMISRTPEVTCVVVDVSQEDPEVQFNWYVDGVEVHNAKTKPREEQFNSTYRVVSVLTVLHQDWLNGKEYKCKVSNKGLASSIEKTISKAKGQPREPQVCTLPPSQEEMTKNQVSLSCAVKGFYPSDIAVEWESNGQPENNYKTTPPVLDSDGSFFLVSKLTVDKSRWQEGNVFSCSVMHEALHNHYTQKSLSLSLGK

SEQ ID NO: 83 - DNA, 1347 bp, Homo sapiens
  source 1..1347: mol_type = other DNA
caggttcagctggtgcagtctggcagcgagctgaagaaacctggcgcctctgtgaaggtgtcctgcaaggctagcggctacatcttcaccaacttcggcatgaactgggtccgagaggctcctggacagggactcgaatggatgggctggatcaacacctacaccggcgagcagatctacgccgatggcttcacaggcagattcgtgttcagcctggacaccagcgccagcacagcttacctgcagatcagctctctgaaggccgaggataccgccgtgtacttctgtgccagaggcgagatctactacggctacgacgtgggctttgtgtactggggccagggaacactggtcaccgttagctctgctagcaccaagggccccagcgtgttccccctggccccttgcagcagaagcaccagcgagagcacagccgccctgggctgcctggtgaaggactacttccccgagcccgtgaccgtgtcctggaacagcggcgctctgaccagcggcgtgcataccttccccgccgtgctccagagcagcggactgtactccctgagcagcgtggtgaccgtgccttccagcagcctgggcaccaagacctacacctgcaacgtggaccacaagcccagcaacaccaaggtggacaagagagtggagagcaagtacggccctccctgccccccttgccctgcccccgagttcgagggcggacctagcgtgttcctgttcccccccaagcccaaggacaccctgatgatcagcagaacccccgaggtgacctgcgtggtggtggacgtgtcccaggaggaccccgaggtccagtttaattggtacgtggacggcgtggaagtgcataacgccaagaccaagcccagagaggagcagttcaacagcacctacagagtggtgtccgtgctgaccgtgctgcaccaggactggctgaacggcaaggaatacaagtgcaaggtctccaacaagggcctggccagcagcatcgagaagaccatcagcaaggccaagggccagccacgggagccccaggtctgcaccctgccacctagccaagaggagatgaccaagaaccaggtgtccctgagctgtgccgtgaaaggcttctatcccagcgatatcgccgtggagtgggagagcaacggccagcccgagaacaactacaagaccaccccccctgtgctggacagcgacggcagcttcttcctggtttccaagctgaccgtggacaagtccagatggcaggagggcaacgtcttcagctgctccgtgatgcacgaggccctgcacaaccactacacccagaagtccctgagcctgagcctgggcaag

SEQ ID NO: 84 - protein, 218 aa, Homo sapiens
DIVLTQSPASLAVSPGQRATITCRASKSVTTSGYSYIHWYQKKPGQPPKLLIYLASDLEAGVPARFSGSGSGTDFTLTINPVEAEDTANYYCQHSRELPWTFGQGTKVEIKRTVAAPSVFIFPPSDEQLKSGTASVVCLLNNFYPREAKVQWKVDNALQSGNSQESVTEQDSKDSTYSLSSTLTLSKADYEKHKVYACEVTHQGLSSPVTKSFNRGEC

SEQ ID NO: 85 - DNA, 654 bp, Homo sapiens
  source 1..654: mol_type = other DNA
gacatcgtgctgacacagagccctgcttctctggctgtgtctcctggccagagagccaccatcacctgtagagccagcaagagcgtgaccaccagcggctactcttacatccactggtatcagaagaagcccggccagcctcctaagctgctgatctacctggccagcgatctggaagctggcgtgccagctagattttctggcagcggctctggcaccgacttcaccctgacaatcaaccccgtggaagccgaagacaccgccaactactactgccagcacagcagagagctgccctggacatttggccagggcaccaaggtggaaatcaagcgaactgtggctgcaccatctgtcttcatcttcccgccatctgatgagcagttgaaatctggaactgcctctgttgtgtgcctgctgaataacttctatcccagagaggccaaagtacagtggaaggtggataacgccctccaatcgggtaactcccaggagagtgtcacagagcaggacagcaaggacagcacctacagcctcagcagcaccctgacgctgagcaaagcagactacgagaaacacaaagtctacgcctgcgaagtcacccatcagggcctgagctcgcccgtcacaaagagcttcaacaggggagagtgt

SEQ ID NO: 86 - protein, 449 aa, Homo sapiens; identical to SEQ ID NO: 82

SEQ ID NO: 87 - DNA, 1347 bp, Homo sapiens; identical to SEQ ID NO: 83
  source 1..1347: mol_type = other DNA

SEQ ID NO: 88 - protein, 219 aa, Homo sapiens
DVVMTQSPLSLPVTPGEPASISCRSSQSIVHSNGNTYLEWYLKKPGQSPQLLIYKVSNRFSGVPDRFSGSGSGTDFTLKISRVEAEDVGVYFCLQVTHVPLTFGQGTKLEIKRTVAAPSVFIFPPSDEQLKSGTASVVCLLNNFYPREAKVQWKVDNALQSGNSQESVTEQDSKDSTYSLSSTLTLSKADYEKHKVYACEVTHQGLSSPVTKSFNRGEC

SEQ ID NO: 89 - DNA, 657 bp, Homo sapiens
  source 1..657: mol_type = other DNA
gacgtggtcatgacacagagccctctgagcctgcctgtgacacctggcgaacctgccagcatcagctgtagaagcagccagagcatcgtgcacagcaacggcaacacatacctggagtggtatctgaagaagcccggccagtctcctcagctgctgatctacaaggtgtccaacagattcagcggcgtgcccgacagattctctggctctggatctggcaccgacttcaccctgaagatctccagagtggaagccgaggacgtgggcgtgtacttctgtctccaggtcacacacgtgcccctgacatttggccagggcaccaagctggaaatcaagcgaactgtggctgcaccatctgtcttcatcttcccgccatctgatgagcagttgaaatctggaactgcctctgttgtgtgcctgctgaataacttctatcccagagaggccaaagtacagtggaaggtggataacgccctccaatcgggtaactcccaggagagtgtcacagagcaggacagcaaggacagcacctacagcctcagcagcaccctgacgctgagcaaagcagactacgagaaacacaaagtctacgcctgcgaagtcacccatcagggcctgagctcgcccgtcacaaagagcttcaacaggggagagtgt

SEQ ID NO: 90 - protein, 442 aa, Homo sapiens
QVQLVQSGAEVKKPGSSVKVSCKASGYTFADYEIHWVREAPGQGLEWMGAIHPGSGGTAYAQKFQGRVTLTADESSTTAYMELSSLRSEDTAVYYCTRYYSFAYWGQGTLVTVSSASTKGPSVFPLAPCSRSTSESTAALGCLVKDYFPEPVTVSWNSGALTSGVHTFPAVLQSSGLYSLSSVVTVPSSSLGTKTYTCNVDHKPSNTKVDKRVESKYGPPCPPCPAPEFEGGPSVFLFPPKPKDTLMISRTPEVTCVVVDVSQEDPEVQFNWYVDGVEVHNAKTKPREEQFNSTYRVVSVLTVLHQDWLNGKEYKCKVSNKGLASSIEKTISKAKGQPREPQVCTLPPSQEEMTKNQVSLSCAVKGFYPSDIAVEWESNGQPENNYKTTPPVLDSDGSFFLVSKLTVDKSRWQEGNVFSCSVMHEALHNHYTQKSLSLSLGK

SEQ ID NO: 91 - DNA, 1326 bp, Homo sapiens
  source 1..1326: mol_type = other DNA
caggttcagctggttcagtctggcgccgaagtgaagaaacctggcagcagcgtgaaggtgtcctgcaaggctagcggctacaccttcgccgactacgagatccactgggtccgagaggctccaggacagggacttgaatggatgggcgctatccatcctggctctggcggcacagcttacgcccagaaattccagggcagagtgaccctgaccgccgacgagtctagcaccaccgcctacatggaactgagcagcctgagaagcgaggacaccgccgtgtactactgcacccggtactacagcttcgcctactggggacagggaaccctggtcacagtcagctctgctagcaccaagggccccagcgtgttccccctggccccttgcagcagaagcaccagcgagagcacagccgccctgggctgcctggtgaaggactacttccccgagcccgtgaccgtgtcctggaacagcggcgctctgaccagcggcgtgcataccttccccgccgtgctccagagcagcggactgtactccctgagcagcgtggtgaccgtgccttccagcagcctgggcaccaagacctacacctgcaacgtggaccacaagcccagcaacaccaaggtggacaagagagtggagagcaagtacggccctccctgccccccttgccctgcccccgagttcgagggcggacctagcgtgttcctgttcccccccaagcccaaggacaccctgatgatcagcagaacccccgaggtgacctgcgtggtggtggacgtgtcccaggaggaccccgaggtccagtttaattggtacgtggacggcgtggaagtgcataacgccaagaccaagcccagagaggagcagttcaacagcacctacagagtggtgtccgtgctgaccgtgctgcaccaggactggctgaacggcaaggaatacaagtgcaaggtctccaacaagggcctggccagcagcatcgagaagaccatcagcaaggccaagggccagccacgggagccccaggtctgcaccctgccacctagccaagaggagatgaccaagaaccaggtgtccctgagctgtgccgtgaaaggcttctatcccagcgatatcgccgtggagtgggagagcaacggccagcccgagaacaactacaagaccaccccccctgtgctggacagcgacggcagcttcttcctggtttccaagctgaccgtggacaagtccagatggcaggagggcaacgtcttcagctgctccgtgatgcacgaggccctgcacaaccactacacccagaagtccctgagcctgagcctgggcaag

SEQ ID NO: 92 - protein, 219 aa, Homo sapiens
DVVMTQSPLSLPVTPGEPASISCRSSQSIVHSNGNTYLEWYLKKPGQSPQLLIYKVSNRFSGVPDRFSGSGSGTDFTLKISRVEAEDVGVYFCLQVTHVPLTFGQGTKLEIKRTVAAPSVFIFPPSDKKLKSGTASVVCLLNNFYPREAKVQWKVDNALQSGNSQESVTEQDSKDSTYSLSSTLTLSKADYEKHKVYACEVTHQGLSSPVTKSFNRGEC

SEQ ID NO: 93 - DNA, 657 bp, Homo sapiens
  source 1..657: mol_type = other DNA
gacgtggtcatgacacagagccctctgagcctgcctgtgacacctggcgaacctgccagcatcagctgtagaagcagccagagcatcgtgcacagcaacggcaacacatacctggagtggtatctgaagaagcccggccagtctcctcagctgctgatctacaaggtgtccaacagattcagcggcgtgcccgacagattctctggctctggatctggcaccgacttcaccctgaagatctccagagtggaagccgaggacgtgggcgtgtacttctgtctccaggtcacacacgtgcccctgacatttggccagggcaccaagctggaaatcaagcgaactgtggctgcaccatctgtcttcatcttcccgccatctgataagaaattgaaatctggaactgcctctgttgtgtgcctgctgaataacttctatcccagagaggccaaagtacagtggaaggtggataacgccctccaatcgggtaactcccaggagagtgtcacagagcaggacagcaaggacagcacctacagcctcagcagcaccctgacgctgagcaaagcagactacgagaaacacaaagtctacgcctgcgaagtcacccatcagggcctgagctcgcccgtcacaaagagcttcaacaggggagagtgt

SEQ ID NO: 94 - protein, 442 aa, Homo sapiens
QVQLVQSGAEVKKPGSSVKVSCKASGYTFADYEIHWVREAPGQGLEWMGAIHPGSGGTAYAQKFQGRVTLTADESSTTAYMELSSLRSEDTAVYYCTRYYSFAYWGQGTLVTVSSASTKGPSVFPLAPCSRSTSESTAALGCLVEDYFPEPVTVSWNSGALTSGVHTFPAVLQSSGLYSLSSVVTVPSSSLGTKTYTCNVDHKPSNTKVDERVESKYGPPCPPCPAPEFEGGPSVFLFPPKPKDTLMISRTPEVTCVVVDVSQEDPEVQFNWYVDGVEVHNAKTKPREEQFNSTYRVVSVLTVLHQDWLNGKEYKCKVSNKGLASSIEKTISKAKGQPREPQVCTLPPSQEEMTKNQVSLSCAVKGFYPSDIAVEWESNGQPENNYKTTPPVLDSDGSFFLVSKLTVDKSRWQEGNVFSCSVMHEALHNHYTQKSLSLSLGK

SEQ ID NO: 95 - DNA, 1326 bp, Homo sapiens
  source 1..1326: mol_type = other DNA
caggttcagctggttcagtctggcgccgaagtgaagaaacctggcagcagcgtgaaggtgtcctgcaaggctagcggctacaccttcgccgactacgagatccactgggtccgagaggctccaggacagggacttgaatggatgggcgctatccatcctggctctggcggcacagcttacgcccagaaattccagggcagagtgaccctgaccgccgacgagtctagcaccaccgcctacatggaactgagcagcctgagaagcgaggacaccgccgtgtactactgcacccggtactacagcttcgcctactggggacagggaaccctggtcacagtcagctctgctagcaccaagggccccagcgtgttccccctggccccttgcagcagaagcaccagcgagagcacagccgccctgggctgcctggtggaggactacttccccgagcccgtgaccgtgtcctggaacagcggcgctctgaccagcggcgtgcataccttccccgccgtgctccagagcagcggactgtactccctgagcagcgtggtgaccgtgccttccagcagcctgggcaccaagacctacacctgcaacgtggaccacaagcccagcaacaccaaggtggacgagagagtggagagcaagtacggccctccctgccccccttgccctgcccccgagttcgaaggcggacctagcgtgttcctgttcccccccaagcccaaggacaccctgatgatcagcagaacccccgaggtgacctgcgtggtggtggacgtgtcccaggaggaccccgaggtccagtttaattggtacgtggacggcgtggaagtgcataacgccaagaccaagcccagagaggagcagttcaacagcacctacagagtggtgtccgtgctgaccgtgctgcaccaggactggctgaacggcaaggaatacaagtgcaaggtctccaacaagggcctggccagcagcatcgagaagaccatcagcaaggccaagggccagccacgggagccccaggtctgcaccctgccacctagccaagaggagatgaccaagaaccaggtgtccctgagctgtgccgtgaaaggcttctatcccagcgatatcgccgtggagtgggagagcaacggccagcccgagaacaactacaagaccaccccccctgtgctggacagcgacggcagcttcttcctggtttccaagctgaccgtggacaagtccagatggcaggagggcaacgtcttcagctgctccgtgatgcacgaggccctgcacaaccactacacccagaagtccctgagcctgagcctgggcaag